European Patent Specification EP 3 337 515 B1, published March 13, 2024. Title: COMPOUNDS AND METHODS FOR TRANS-MEMBRANE DELIVERY OF MOLECULES. Applicant: Aposense LTD. ZIV, Ilan. The sequence listing filed with the application follows.

SEQUENCE LISTING (10 sequences)

SEQ ID NO: 1 - DNA, 27 bp, Artificial Sequence
  Single strand DNA oligonucleotide
  misc_feature (1)..(1): C is attached to MNM-TT-iCy3
cggtggtgcagatgaacttcagggtca

SEQ ID NO: 2 - DNA, 29 bp, Artificial Sequence
  Single strand DNA oligonucleotide
  misc_feature (1)..(1): T is attached to MNM
tgaccctgaagttcatctgcaccaccgaa

SEQ ID NO: 3 - DNA, 27 bp, Artificial Sequence
  Single strand DNA oligonucleotide
  misc_feature (1)..(1): C is attached to Apo-si-11-TT-iCy3
cggtggtgcagatgaacttcagggtca

SEQ ID NO: 4 - DNA, 29 bp, Artificial Sequence
  Single strand DNA oligonucleotide
  misc_feature (1)..(1): T is attached to Apo-si-11
tgaccctgaagttcatctgcaccaccgaa

SEQ ID NO: 5 - RNA, 25 nt, Artificial Sequence
  Artificial short sequence
acccugaaguucaucugcaccaccg

SEQ ID NO: 6 - RNA, 27 nt, Artificial Sequence
  Artificial short sequence
cgguggugcagaugaacuucaggguca

SEQ ID NO: 7 - RNA, 27 nt, Artificial Sequence
  Artificial short sequence
  misc_feature (1)..(1): C is attached to Apo-Si-S-S
cgguggugcagaugaacuucaggguca

SEQ ID NO: 8 - RNA, 25 nt, Artificial Sequence
  Artificial short sequence
  misc_feature (1)..(1): A is attached to Apo-Si-S-S
acccugaaguucaucugcaccaccg

SEQ ID NO: 9 - DNA, 25 bp, Artificial Sequence
  Single strand DNA oligonucleotide
  misc_feature (1)..(1): C is attached to MNM/TT/iCy3
cggtggcagatgaacttcagggtca

SEQ ID NO: 10 - DNA, 27 bp, Artificial Sequence
  Single strand DNA oligonucleotide
  misc_feature (1)..(1): T is attached to MNM
tgaccctgaagttcatctgccaccgaa